European Patent Application EP 4 353 260 A1, published April 17, 2024. Title: Enhancement of innate immune response. Applicant: Kyoto University. The sequence listing filed with the application follows.

SEQUENCE LISTING (15 sequences)

SEQ ID NO: 1 - DNA, 24 bp, Artificial Sequence
  designed for the sequence adjacent to the OAS1 exon 5 splice donor (oAM685)
cugcuggugagaccuccugcuucc

SEQ ID NO: 2 - DNA, 20 bp, Artificial Sequence
  Forward primer for ACTB (oAM13)
ccaaccgcgagaagatgacc

SEQ ID NO: 3 - DNA, 20 bp, Artificial Sequence
  Reverse primer for ACTB (oAM14)
agcttctccttaatgtcacg

SEQ ID NO: 4 - DNA, 19 bp, Artificial Sequence
  Forward primer for OAS1 (oAM674)
ggttggaggcagctggcac

SEQ ID NO: 5 - DNA, 20 bp, Artificial Sequence
  Reverse primer for OAS1 (oAM675)
ccagctatatgtctcaagct

SEQ ID NO: 6 - DNA, 20 bp, Artificial Sequence
  Reverse primer for OAS1 (oAM676)
ctggcattcagaggatggtg

SEQ ID NO: 7 - DNA, 20 bp, Artificial Sequence
  Reverse primer for OAS1 (oAM677)
ctgcctccctaagcaacctg

SEQ ID NO: 8 - DNA, 20 bp, Artificial Sequence
  Reverse primer for OAS1 (oAM678)
ccatttccaccacttgttag

SEQ ID NO: 9 - DNA, 20 bp, Artificial Sequence
  Forward primer for IFNB1 (oAM700)
cagtgtcagaagctcctgtg

SEQ ID NO: 10 - DNA, 20 bp, Artificial Sequence
  Reverse primer for IFNB1 (oAM701)
atctgatgatagacattagc

SEQ ID NO: 11 - DNA, 12 bp, Homo sapiens
cccuuucaggcu

SEQ ID NO: 12 - DNA, 11 bp, Artificial Sequence
  5' end of U1snRNP
  misc_feature (5)..(6): n is p (pseudouridine)
auacnnaccug

SEQ ID NO: 13 - DNA, 27 bp, Homo sapiens
gcuggugagaccuccugcuuccucccu

SEQ ID NO: 14 - DNA, 15 bp, Homo sapiens
cctttcaagctgaaa

SEQ ID NO: 15 - DNA, 15 bp, Homo sapiens
cctttcaggctgaaa